European Patent Application EP 4 667 491 A1, published December 24, 2025. Title: ANTI-CNTN4 ANTIBODY AND ITS USE. Applicant: GENOME AND COMPANY. The sequence listing filed with the application follows.

SEQUENCE LISTING (67 sequences)

SEQ ID NO: 1 - protein, 5 aa, synthetic construct
SFNMF

SEQ ID NO: 2 - protein, 8 aa, synthetic construct
SGSSGSYG

SEQ ID NO: 3 - protein, 8 aa, synthetic construct
SGRSGSYG

SEQ ID NO: 4 - protein, 17 aa, synthetic construct
EISGGGGSTWYAPAVKG

SEQ ID NO: 5 - protein, 7 aa, synthetic construct
DNTNRPS

SEQ ID NO: 6 - protein, 14 aa, synthetic construct
SRDTWSYGAATIDA

SEQ ID NO: 7 - protein, 9 aa, synthetic construct
GGYDGSTDV

SEQ ID NO: 8 - protein, 14 aa, synthetic construct
SIDTWSYGAATIDA

SEQ ID NO: 9 - protein, 14 aa, synthetic construct
SAFTWSYGAATIDA

SEQ ID NO: 10 - protein, 14 aa, synthetic construct
SADTWSYGAASIDA

SEQ ID NO: 11 - protein, 14 aa, synthetic construct
SADTWSYGAADIDA

SEQ ID NO: 12 - protein, 14 aa, synthetic construct
SADTWSYGAATIRA

SEQ ID NO: 13 - protein, 14 aa, synthetic construct
SADTWSYGAATILA

SEQ ID NO: 14 - protein, 14 aa, synthetic construct
SADTWSYGAATISA

SEQ ID NO: 15 - protein, 14 aa, synthetic construct
SADTWSYGAATIAA

SEQ ID NO: 16 - protein, 14 aa, synthetic construct
SADTWSYGAATIGA

SEQ ID NO: 17 - protein, 14 aa, synthetic construct
SADTWSYGAATIQA

SEQ ID NO: 18 - protein, 14 aa, synthetic construct
SADTWSYGAATIDA

SEQ ID NO: 19 - protein, 9 aa, synthetic construct
GGYRGSTDV

SEQ ID NO: 20 - protein, 9 aa, synthetic construct
GGYWGSTDV

SEQ ID NO: 21 - protein, 14 aa, synthetic construct
SAFTWSYGAADIAA

SEQ ID NO: 22 - protein, 14 aa, synthetic construct
SADTWSYGAADISA

SEQ ID NO: 23 - protein, 14 aa, synthetic construct
SRDTWSYGAADIAA

SEQ ID NO: 24 - protein, 14 aa, synthetic construct
SADTWSYGAADIAA

SEQ ID NO: 25 - protein, 14 aa, synthetic construct
SADTWSYGAADIQA

SEQ ID NO: 26 - protein, 14 aa, synthetic construct
SAFTWSYGAADIDA

SEQ ID NO: 27 - protein, 14 aa, synthetic construct
SAFTWSYGAADISA

SEQ ID NO: 28 - protein, 14 aa, synthetic construct
SADTWSYGAASISA

SEQ ID NO: 29 - protein, 14 aa, synthetic construct
SRDTWSYGAADIDA

SEQ ID NO: 30 - protein, 14 aa, synthetic construct
SAFTWSYGAASIQA

SEQ ID NO: 31 - protein, 14 aa, synthetic construct
SADTWSYGAASIAA

SEQ ID NO: 32 - protein, 14 aa, synthetic construct
SRFTWSYGAADISA

SEQ ID NO: 33 - protein, 14 aa, synthetic construct
SAFTWSYGAATISA

SEQ ID NO: 34 - protein, 14 aa, synthetic construct
SRFTWSYGAASIAA

SEQ ID NO: 35 - protein, 14 aa, synthetic construct
SAYTWSYGAATIYA

SEQ ID NO: 36 - protein, 123 aa, synthetic construct
EVQLLESGGGLVQPGGSLRLSCAASGFTFSSFNMFWVRQAPGKGLEWVAEISGGGGSTWYAPAVKGRFTISRDNSKNTLYLQMNSLRAEDTAVYYCAKSRDTWSYGAATIDAWGQGTLVTVSS

SEQ ID NO: 37 - protein, 101 aa, synthetic construct
ELTQDPAVSVALGQTVRITCSGSSGSYGWYQQKPGQAPVLVIYDNTNRPSGIPDRFSGSSSGNTASLTITGAQAEDEADYYCGGYDGSTDVFGGGTKLTVL

SEQ ID NO: 38 - protein, 123 aa, synthetic construct
EVQLLESGGGLVQPGGSLRLSCAASGFTFSSFNMFWVRQAPGKGLEWVAEISGGGGSTWYAPAVKGRFTISRDNSKNTLYLQMNSLRAEDTAVYYCAKSIDTWSYGAATIDAWGQGTLVTVSS

SEQ ID NO: 39 - protein, 123 aa, synthetic construct
EVQLLESGGGLVQPGGSLRLSCAASGFTFSSFNMFWVRQAPGKGLEWVAEISGGGGSTWYAPAVKGRFTISRDNSKNTLYLQMNSLRAEDTAVYYCAKSAFTWSYGAATIDAWGQGTLVTVSS

SEQ ID NO: 40 - protein, 123 aa, synthetic construct
EVQLLESGGGLVQPGGSLRLSCAASGFTFSSFNMFWVRQAPGKGLEWVAEISGGGGSTWYAPAVKGRFTISRDNSKNTLYLQMNSLRAEDTAVYYCAKSADTWSYGAASIDAWGQGTLVTVSS

SEQ ID NO: 41 - protein, 123 aa, synthetic construct
EVQLLESGGGLVQPGGSLRLSCAASGFTFSSFNMFWVRQAPGKGLEWVAEISGGGGSTWYAPAVKGRFTISRDNSKNTLYLQMNSLRAEDTAVYYCAKSADTWSYGAADIDAWGQGTLVTVSS

SEQ ID NO: 42 - protein, 123 aa, synthetic construct
EVQLLESGGGLVQPGGSLRLSCAASGFTFSSFNMFWVRQAPGKGLEWVAEISGGGGSTWYAPAVKGRFTISRDNSKNTLYLQMNSLRAEDTAVYYCAKSADTWSYGAATIRAWGQGTLVTVSS

SEQ ID NO: 43 - protein, 123 aa, synthetic construct
EVQLLESGGGLVQPGGSLRLSCAASGFTFSSFNMFWVRQAPGKGLEWVAEISGGGGSTWYAPAVKGRFTISRDNSKNTLYLQMNSLRAEDTAVYYCAKSADTWSYGAATILAWGQGTLVTVSS

SEQ ID NO: 44 - protein, 123 aa, synthetic construct
EVQLLESGGGLVQPGGSLRLSCAASGFTFSSFNMFWVRQAPGKGLEWVAEISGGGGSTWYAPAVKGRFTISRDNSKNTLYLQMNSLRAEDTAVYYCAKSADTWSYGAATISAWGQGTLVTVSS

SEQ ID NO: 45 - protein, 123 aa, synthetic construct
EVQLLESGGGLVQPGGSLRLSCAASGFTFSSFNMFWVRQAPGKGLEWVAEISGGGGSTWYAPAVKGRFTISRDNSKNTLYLQMNSLRAEDTAVYYCAKSADTWSYGAATIAAWGQGTLVTVSS

SEQ ID NO: 46 - protein, 123 aa, synthetic construct
EVQLLESGGGLVQPGGSLRLSCAASGFTFSSFNMFWVRQAPGKGLEWVAEISGGGGSTWYAPAVKGRFTISRDNSKNTLYLQMNSLRAEDTAVYYCAKSADTWSYGAATIGAWGQGTLVTVSS

SEQ ID NO: 47 - protein, 123 aa, synthetic construct
EVQLLESGGGLVQPGGSLRLSCAASGFTFSSFNMFWVRQAPGKGLEWVAEISGGGGSTWYAPAVKGRFTISRDNSKNTLYLQMNSLRAEDTAVYYCAKSADTWSYGAATIQAWGQGTLVTVSS

SEQ ID NO: 48 - protein, 123 aa, synthetic construct
EVQLLESGGGLVQPGGSLRLSCAASGFTFSSFNMFWVRQAPGKGLEWVAEISGGGGSTWYAPAVKGRFTISRDNSKNTLYLQMNSLRAEDTAVYYCAKSADTWSYGAATIDAWGQGTLVTVSS

SEQ ID NO: 49 - protein, 101 aa, synthetic construct
ELTQDPAVSVALGQTVRITCSGRSGSYGWYQQKPGQAPVLVIYDNTNRPSGIPDRFSGSSSGNTASLTITGAQAEDEADYYCGGYDGSTDVFGGGTKLTVL

SEQ ID NO: 50 - protein, 101 aa, synthetic construct
ELTQDPAVSVALGQTVRITCSGSSGSYGWYQQKPGQAPVLVIYDNTNRPSGIPDRFSGSSSGNTASLTITGAQAEDEADYYCGGYRGSTDVFGGGTKLTVL

SEQ ID NO: 51 - protein, 101 aa, synthetic construct
ELTQDPAVSVALGQTVRITCSGSSGSYGWYQQKPGQAPVLVIYDNTNRPSGIPDRFSGSSSGNTASLTITGAQAEDEADYYCGGYWGSTDVFGGGTKLTVL

SEQ ID NO: 52 - protein, 123 aa, synthetic construct
EVQLLESGGGLVQPGGSLRLSCAASGFTFSSFNMFWVRQAPGKGLEWVAEISGGGGSTWYAPAVKGRFTISRDNSKNTLYLQMNSLRAEDTAVYYCAKSAFTWSYGAADIAAWGQGTLVTVSS

SEQ ID NO: 53 - protein, 101 aa, synthetic construct
ELTQDPAVSVALGQTVRITCSGRSGSYGWYQQKPGQAPVLVIYDNTNRPSGIPDRFSGSSSGNTASLTITGAQAEDEADYYCGGYWGSTDVFGGGTKLTVL

SEQ ID NO: 54 - protein, 123 aa, synthetic construct
EVQLLESGGGLVQPGGSLRLSCAASGFTFSSFNMFWVRQAPGKGLEWVAEISGGGGSTWYAPAVKGRFTISRDNSKNTLYLQMNSLRAEDTAVYYCAKSADTWSYGAADISAWGQGTLVTVSS

SEQ ID NO: 55 - protein, 123 aa, synthetic construct
EVQLLESGGGLVQPGGSLRLSCAASGFTFSSFNMFWVRQAPGKGLEWVAEISGGGGSTWYAPAVKGRFTISRDNSKNTLYLQMNSLRAEDTAVYYCAKSRDTWSYGAADIAAWGQGTLVTVSS

SEQ ID NO: 56 - protein, 123 aa, synthetic construct
EVQLLESGGGLVQPGGSLRLSCAASGFTFSSFNMFWVRQAPGKGLEWVAEISGGGGSTWYAPAVKGRFTISRDNSKNTLYLQMNSLRAEDTAVYYCAKSADTWSYGAADIAAWGQGTLVTVSS

SEQ ID NO: 57 - protein, 123 aa, synthetic construct
EVQLLESGGGLVQPGGSLRLSCAASGFTFSSFNMFWVRQAPGKGLEWVAEISGGGGSTWYAPAVKGRFTISRDNSKNTLYLQMNSLRAEDTAVYYCAKSADTWSYGAADIQAWGQGTLVTVSS

SEQ ID NO: 58 - protein, 123 aa, synthetic construct
EVQLLESGGGLVQPGGSLRLSCAASGFTFSSFNMFWVRQAPGKGLEWVAEISGGGGSTWYAPAVKGRFTISRDNSKNTLYLQMNSLRAEDTAVYYCAKSAFTWSYGAADIDAWGQGTLVTVSS

SEQ ID NO: 59 - protein, 123 aa, synthetic construct
EVQLLESGGGLVQPGGSLRLSCAASGFTFSSFNMFWVRQAPGKGLEWVAEISGGGGSTWYAPAVKGRFTISRDNSKNTLYLQMNSLRAEDTAVYYCAKSAFTWSYGAADISAWGQGTLVTVSS

SEQ ID NO: 60 - protein, 123 aa, synthetic construct
EVQLLESGGGLVQPGGSLRLSCAASGFTFSSFNMFWVRQAPGKGLEWVAEISGGGGSTWYAPAVKGRFTISRDNSKNTLYLQMNSLRAEDTAVYYCAKSADTWSYGAASISAWGQGTLVTVSS

SEQ ID NO: 61 - protein, 123 aa, synthetic construct
EVQLLESGGGLVQPGGSLRLSCAASGFTFSSFNMFWVRQAPGKGLEWVAEISGGGGSTWYAPAVKGRFTISRDNSKNTLYLQMNSLRAEDTAVYYCAKSRDTWSYGAADIDAWGQGTLVTVSS

SEQ ID NO: 62 - protein, 123 aa, synthetic construct
EVQLLESGGGLVQPGGSLRLSCAASGFTFSSFNMFWVRQAPGKGLEWVAEISGGGGSTWYAPAVKGRFTISRDNSKNTLYLQMNSLRAEDTAVYYCAKSAFTWSYGAASIQAWGQGTLVTVSS

SEQ ID NO: 63 - protein, 123 aa, synthetic construct
EVQLLESGGGLVQPGGSLRLSCAASGFTFSSFNMFWVRQAPGKGLEWVAEISGGGGSTWYAPAVKGRFTISRDNSKNTLYLQMNSLRAEDTAVYYCAKSADTWSYGAASIAAWGQGTLVTVSS

SEQ ID NO: 64 - protein, 123 aa, synthetic construct
EVQLLESGGGLVQPGGSLRLSCAASGFTFSSFNMFWVRQAPGKGLEWVAEISGGGGSTWYAPAVKGRFTISRDNSKNTLYLQMNSLRAEDTAVYYCAKSRFTWSYGAADISAWGQGTLVTVSS

SEQ ID NO: 65 - protein, 123 aa, synthetic construct
EVQLLESGGGLVQPGGSLRLSCAASGFTFSSFNMFWVRQAPGKGLEWVAEISGGGGSTWYAPAVKGRFTISRDNSKNTLYLQMNSLRAEDTAVYYCAKSAFTWSYGAATISAWGQGTLVTVSS

SEQ ID NO: 66 - protein, 123 aa, synthetic construct
EVQLLESGGGLVQPGGSLRLSCAASGFTFSSFNMFWVRQAPGKGLEWVAEISGGGGSTWYAPAVKGRFTISRDNSKNTLYLQMNSLRAEDTAVYYCAKSRFTWSYGAASIAAWGQGTLVTVSS

SEQ ID NO: 67 - protein, 123 aa, synthetic construct
EVQLLESGGGLVQPGGSLRLSCAASGFTFSSFNMFWVRQAPGKGLEWVAEISGGGGSTWYAPAVKGRFTISRDNSKNTLYLQMNSLRAEDTAVYYCAKSAYTWSYGAATIYAWGQGTLVTVSS